European Patent Specification EP 3 628 334 B1, published June 28, 2023. Title: GENE THERAPY FOR RETINITIS PIGMENTOSA. Applicant: Catherine O'Riordan Matthew Adamowicz. Application Not Yet Assigned. The sequence listing filed with the application follows.

SEQUENCE LISTING (30 sequences)

SEQ ID NO: 1 - DNA, 88 bp, Homo sapiens
aactgccctcaaggagcttacaatctagctgggggtaaatgacttgcacatgaacacaactagactgtgagcttctagagggcaggga

SEQ ID NO: 2 - protein, 348 aa, Homo sapiens [sequence omitted]

SEQ ID NO: 3 - DNA, 1044 bp, Homo sapiens
atgaatggcacagaaggccctaacttctacgtgcccttctccaatgcgacgggtgtggtacgcagccccttcgagtacccacagtactacctggctgagccatggcagttctccatgctggccgcctacatgtttctgctgatcgtgctgggcttccccatcaacttcctcacgctctacgtcaccgtccagcacaagaagctgcgcacgcctctcaactacatcctgctcaacctagccgtggctgacctcttcatggtcctaggtggcttcaccagcaccctctacacctctctgcatggatacttcgtcttcgggcccacaggatgcaatttggagggcttctttgccaccctgggcggtgaaattgccctgtggtccttggtggtcctggccatcgagcggtacgtggtggtgtgtaagcccatgagcaacttccgcttcggggagaaccatgccatcatgggcgttgccttcacctgggtcatggcgctggcctgcgccgcacccccactcgccggctggtccaggtacatccccgagggcctgcagtgctcgtgtggaatcgactactacacgctcaagccggaggtcaacaacgagtcttttgtcatctacatgttcgtggtccacttcaccatccccatgattatcatctttttctgctatgggcagctcgtcttcaccgtcaaggaggccgctgcccagcagcaggagtcagccaccacacagaaggcagagaaggaggtcacccgcatggtcatcatcatggtcatcgctttcctgatctgctgggtgccctacgccagcgtggcattctacatcttcacccaccagggctccaacttcggtcccatcttcatgaccatcccagcgttctttgccaagagcgccgccatctacaaccctgtcatctatatcatgatgaacaagcagttccggaactgcatgctcaccaccatctgctgcggcaagaacccactgggtgacgatgaggcctctgctaccgtgtccaagacggagacgagccaggtggccccggcc

SEQ ID NO: 4 - DNA, 2768 bp, Homo sapiens
agagtcatccagctggagccctgagtggctgagctcaggccttcgcagcattcttgggtgggagcagccacgggtcagccacaagggccacagccatgaatggcacagaaggccctaacttctacgtgcccttctccaatgcgacgggtgtggtacgcagccccttcgagtacccacagtactacctggctgagccatggcagttctccatgctggccgcctacatgtttctgctgatcgtgctgggcttccccatcaacttcctcacgctctacgtcaccgtccagcacaagaagctgcgcacgcctctcaactacatcctgctcaacctagccgtggctgacctcttcatggtcctaggtggcttcaccagcaccctctacacctctctgcatggatacttcgtcttcgggcccacaggatgcaatttggagggcttctttgccaccctgggcggtgaaattgccctgtggtccttggtggtcctggccatcgagcggtacgtggtggtgtgtaagcccatgagcaacttccgcttcggggagaaccatgccatcatgggcgttgccttcacctgggtcatggcgctggcctgcgccgcacccccactcgccggctggtccaggtacatccccgagggcctgcagtgctcgtgtggaatcgactactacacgctcaagccggaggtcaacaacgagtcttttgtcatctacatgttcgtggtccacttcaccatccccatgattatcatctttttctgctatgggcagctcgtcttcaccgtcaaggaggccgctgcccagcagcaggagtcagccaccacacagaaggcagagaaggaggtcacccgcatggtcatcatcatggtcatcgctttcctgatctgctgggtgccctacgccagcgtggcattctacatcttcacccaccagggctccaacttcggtcccatcttcatgaccatcccagcgttctttgccaagagcgccgccatctacaaccctgtcatctatatcatgatgaacaagcagttccggaactgcatgctcaccaccatctgctgcggcaagaacccactgggtgacgatgaggcctctgctaccgtgtccaagacggagacgagccaggtggccccggcctaagacctgcctaggactctgtggccgactataggcgtctcccatcccctacaccttcccccagccacagccatcccaccaggagcagcgcctgtgcagaatgaacgaagtcacataggctccttaattttttttttttttttaagaaataattaatgaggctcctcactcacctgggacagcctgagaagggacatccaccaagacctactgatctggagtcccacgttccccaaggccagcgggatgtgtgcccctcctcctcccaactcatctttcaggaacacgaggattcttgctttctggaaaagtgtcccagcttagggataagtgtctagcacagaatggggcacacagtaggtgcttaataaatgctggatggatgcaggaaggaatggaggaatgaatgggaagggagaacatatctatcctctcagaccctcgcagcagcagcaactcatacttggctaatgatatggagcagttgtttttccctccctgggcctcactttcttctcctataaaatggaaatcccagatccctggtcctgccgacacgcagctactgagaagaccaaaagaggtgtgtgtgtgtctatgtgtgtgtttcagcactttgtaaatagcaagaagctgtacagattctagttaatgttgtgaataacatcaattaatgtaactagttaattactatgattatcacctcctgatagtgaacattttgagattgggcattcagatgatggggtttcacccaaccttggggcaggtttttaaaaattagctaggcatcaaggccagaccagggctgggggttgggctgtaggcagggacagtcacaggaatgcagaatgcagtcatcagacctgaaaaaacaacactgggggagggggacggtgaaggccaagttcccaatgagggtgagattgggcctggggtctcacccctagtgtggggccccaggtcccgtgcctccccttcccaatgtggcctatggagagacaggcctttctctcagcctctggaagccacctgctcttttgctctagcacctgggtcccagcatctagagcatggagcctctagaagccatgctcacccgcccacatttaattaacagctgagtccctgatgtcatccttatctcgaagagcttagaaacaaagagtgggaaattccactgggcctaccttccttggggatgttcatgggccccagtttccagtttcccttgccagacaagcccatcttcagcagttgctagtccattctccattctggagaatctgctccaaaaagctggccacatctctgaggtgtcagaattaagctgcctcagtaactgctcccccttctccatataagcaaagccagaagctctagctttacccagctctgcctggagactaaggcaaattgggccattaaaagctcagctcctatgttggtattaacggtggtgggttttgttgctttcacactctatccacaggatagattgaaactgccagcttccacctgatccctgaccctgggatggctggattgagcaatgagcagagccaagcagcacagagtcccctggggctagaggtggaggaggcagtcctgggaatgggaaaaacccca

SEQ ID NO: 5 - DNA, 1512 bp, Artificial Sequence
  Synthetic Construct
ggccccagaagcctggtggttgtttgtccttctcaggggaaaagtgaggcggccccttggaggaaggggccgggcagaatgatctaatcggattccaagcagctcaggggattgtctttttctagcaccttcttgccactcctaagcgtcctccgtgaccccggctgggatttagcctggtgctgtgtcagccccggtctcccaggggcttcccagtggtccccaggaaccctcgacagggcccggtctctctcgtccagcaagggcagggacgggccacaggccaagggcggagtcgctgcgacgctgccttcgccccgtgccccgctccgccgccgcctcgcgccgcccgccccggctctgactgaccgcgttactcccacaggtgagcgggcgggacggcccttctcctccgggctgtaattagcgcttggtttaatgacggcttgtttcttttctgtggctgcgtgaaagccttgaggggctccgggagggccctttgtgcggggggagcggctcggggggtgcgtgcgtgtgtgtgtgcgtggggagcgccgcgtgcggctccgcgctgcccggcggctgtgagcgctgcgggcgcggcgcggggctttgtgcgctccgcagtgtgcgcgaggggagcgcggccgggggcggtgccccgcggtgcggggggggctgcgaggggaacaaaggctgcgtgcggggtgtgtgcgtgggggggtgagcagggggtgtgggcgcgtcggtcgggctgcaaccccccctgcacccccctccccgagttgctgagcacggcccggcttcgggtgcggggctccgtacggggcgtggcgcggggctcgccgtgccgggcggggggtggcggcaggtgggggtgccgggcggggcggggccgcctcgggccggggagggctcgggggaggggcgcggcggcccccggagcgccggcggctgtcgaggcgcggcgagccgcagccattgccttttatggtaatcgtgcgagagggcgcagggacttcctttgtcccaaatctgtgcggagccgaaatctgggaggcgccgccgcaccccctctagcgggcgcggggcgaagcggtgcggcgccggcaggaaggaaatgggcggggagggccttcgtgcgtcgccgcgccgccgtccccttctccctctccagcctcggggctgtccgcggggggacggctgccttcgggggggacggggcagggcggggttcggcttctggcgtgtgaccggcggctctagagcctctgctaaccatgttcatgccttcttctttttcctacagctcctgggcaacgtgctggttattgtgctgtctcatcattttggcaaagaattcttcgaaagatcctggaggcttgctgaaggctgtatgctgaaggagcttacaatctagctggggttttggccactgactgaccccagctagtgtaagctccttcaggacacaaggcctgttactagcactcacatggaacaaatggccca

SEQ ID NO: 6 - DNA, 3444 bp, Artificial Sequence
  Synthetic Construct
caatctcccagatgctgattcagccaggaactagttattaatagtaatcaattacggggtcattagttcatagcccatatatggagttccgcgttacataacttacggtaaatggcccgcctggctgaccgcccaacgacccccgcccattgacgtcaataatgacgtatgttcccatagtaacgccaatagggactttccattgacgtcaatgggtggagtatttacggtaaactgcccacttggcagtacatcaagtgtatcatatgccaagtacgccccctattgacgtcaatgacggtaaatggcccgcctggcattatgcccagtacatgaccttatgggactttcctacttggcagtacatctacgtattagtcatcgctattaccacaaatagttatcgagccgctgagccggggggcggggggtgtgagactggaggcgatggacggagctgacggcacacacagctcagatctgtcaagtgagccattgtcagggcttggggactggataagtcagggggtctcctgggaagagatgggataggtgagttcaggaggagacattgtcaactggagccatgtggagaagtgaatttagggcccaaaggttccagtcgcagcctgaggccaccagactgacatggggaggaattcccagaggactctggggcagacaagatgagacaccctttcctttctttacctaagggcctccacccgatgtcaccttggcccctctgcaagccaattaggccccggtggcagcagtgggattagcgttagtatgatatctcgcggatgctgaatcagcctctggcttagggagagaaggtcactttataagggtctggggggggtcagtgcctggagttgcgctgtgggagccgtcagtggctgagctcaagaggtaagggtttaagggatggttggttggtggggtattaatgtttaattacctgttttacaggcctgaaatcacttggttttaggttggtacatctgcagaattcagccaccaccggcacaatgaatggcacagaaggccctaacttctacgtgcccttctccaatgcgacgggtgtggtacgcagccccttcgagtacccacagtactacctggctgagccatggcagttctccatgctggccgcctacatgtttctgctgatcgtgctgggcttccccatcaacttcctcacgctctacgtcaccgtccagcacaagaagctgcgcacgcctctcaactacatcctgctcaacctagccgtggctgacctcttcatggtcctaggtggcttcaccagcaccctctacacctctctgcatggatacttcgtcttcgggcccacaggatgcaatttggagggcttctttgccaccctgggcggtgaaattgccctgtggtccttggtggtcctggccatcgagcggtacgtggtggtgtgtaagcccatgagcaacttccgcttcggggagaaccatgccatcatgggcgttgccttcacctgggtcatggcgctggcctgcgccgcacccccactcgccggctggtccaggtacatccccgagggcctgcagtgctcgtgtggaatcgactactacacgctcaagccggaggtcaacaacgagtcttttgtcatctacatgttcgtggtccacttcaccatccccatgattatcatctttttctgctatgggcagctcgtcttcaccgtcaaggaggccgctgcccagcagcaggagtcagccaccacacagaaggcagagaaggaggtcacccgcatggtcatcatcatggtcatcgctttcctgatctgctgggtgccctacgccagcgtggcattctacatcttcacccaccagggctccaacttcggtcccatcttcatgaccatcccagcgttctttgccaagagcgccgccatctacaaccctgtcatctatatcatgatgaacaagcagttccggaactgcatgctcaccaccatctgctgcggcaagaacccactgggtgacgatgaggcctctgctaccgtgtccaagacggagacgagccaggtggccccggcctaaccaagaaagcttaagtttgtgtcccggcttagggctaaatgtctaggacagaatggaacacatagtagctgattaataaatgctagctggatgaagggaggaatgagtgactgactgagtggatatatgagtgaagggattaatggaagggaacatggatgtcctcaggtgcccaacctggcagatccagtcatgtctggctggaatctataagcagttttacatacctgccctgagctttattgcggtagtttatcacagttaaattgctaacgcagtcagtgcttctgacacaacagtctcgaacttaagctgcagtgactctcttaaggtagccttgcagaagttggtcgtgaggcactgggcaggtaagtatcaaggttacaagacaggtttaaggagaccaatagaaactgggcttgtcgagacagagaaaaacctaacccccatggttggcgagggactgctgtgtgtgaaatggtaactgccctcaaggagcttacaatctagctgggggtaaatgacttgcacatgaacacaactagactgtgagcttctagagggcagggaccttaccctagtcatctctcttctcaccctgcacaccctccctgagggatctcatgactcttgcgtttctgataggcacctattggtcttactgacatccactttgcctttctctccacaggtgtccactcccagttcacaccggcacaatgaatggcacagaaggccctaacttctacgtgcccttctccaatgcgacgggtgtggtacgcagccccttcgagtacccacagtcagagataaatgacagtgacagcaacgtgagctgcagcccttaggactgagaaagcatcgagaccaggggtctccggcaaggcctaggtcctcccttcagtatggaaaccttgcctcatgtctctcagcctccttggcctgtggagatccagcccttcctcttggcttctggatacatttgctcttctacaccagcaaccaagtggcaacagttccaggccagtatggagttttagaagccatgccaatatgcccaccttcagggagcagctgagtccttgatgccacccttgttctgaagagttcagaaacacagtgcaagacatgaccaggcctcatccttaggatgctcatggatccagttcttagctcccttgttggatatgctgttttccttggcctttggtcttttctttatcccagagggttttggctttaaggccaacaggaactatggggtaccagaattgagcagcctcagtctgcatccctcctctatagaaccacagctgggccctcagcaggcccaactctgcatggggacagaggcattaaaagc

SEQ ID NO: 7 - DNA, 3014 bp, Artificial Sequence
  Synthetic Construct
gggccccagaagcctggtggttgtttgtccttctcaggggaaaagtgaggcggccccttggaggaaggggccgggcagaatgatctaatcggattccaagcagctcaggggattgtctttttctagcaccttcttgccactcctaagcgtcctccgtgaccccggctgggatttagcctggtgctgtgtcagccccggtctcccaggggcttcccagtggtccccaggaaccctcgacagggcccggtctctctcgtccagcaagggcagggacgggccacaggccaagggcggagtcgctgcgacgctgccttcgccccgtgccccgctccgccgccgcctcgcgccgcccgccccggctctgactgaccgcgttactcccacaggtgagcgggcgggacggcccttctcctccgggctgtaattagcaagaggtaagggtttaagggatggttggttggtggggtattaatgtttaattacctgttttacaggcctgaaatcacttggttttaggttggggatccggtacccaattgccatgggctagcatgcatgagctccctgcagggtttatctgcagaattcagccaccaccggcacaatgaatggcacagaaggccctaacttctacgtgcccttctccaatgcgacgggtgtggtacgcagccccttcgagtacccacagtactacctggctgagccatggcagttctccatgctggccgcctacatgtttctgctgatcgtgctgggcttccccatcaacttcctcacgctctacgtcaccgtccagcacaagaagctgcgcacgcctctcaactacatcctgctcaacctagccgtggctgacctcttcatggtcctaggtggcttcaccagcaccctctacacctctctgcatggatacttcgtcttcgggcccacaggatgcaatttggagggcttctttgccaccctgggcggtgaaattgccctgtggtccttggtggtcctggccatcgagcggtacgtggtggtgtgtaagcccatgagcaacttccgcttcggggagaaccatgccatcatgggcgttgccttcacctgggtcatggcgctggcctgcgccgcacccccactcgccggctggtccaggtacatccccgagggcctgcagtgctcgtgtggaatcgactactacacgctcaagccggaggtcaacaacgagtcttttgtcatctacatgttcgtggtccacttcaccatccccatgattatcatctttttctgctatgggcagctcgtcttcaccgtcaaggaggccgctgcccagcagcaggagtcagccaccacacagaaggcagagaaggaggtcacccgcatggtcatcatcatggtcatcgctttcctgatctgctgggtgccctacgccagcgtggcattctacatcttcacccaccagggctccaacttcggtcccatcttcatgaccatcccagcgttctttgccaagagcgccgccatctacaaccctgtcatctatatcatgatgaacaagcagttccggaactgcatgctcaccaccatctgctgcggcaagaacccactgggtgacgatgaggcctctgctaccgtgtccaagacggagacgagccaggtggccccggcctaaccaagaaagcttaagtttgtgtcccggcttagggctaaatgtctaggacagaatggaacacatagtagctgattaataaatgctagctggatgaagggaggaatgagtgactgactgagtggatatatgagtgaagggattaatggaagggaacatggatgtcctcaggtgcccaacctggcagatccagtcatgtctggctggaatctataagcagttttacatacctgccctgagctttattgcggtagtttatcacagttaaattgctaacgcagtcagtgcttctgacacaacagtctcgaacttaagctgcagtgactctcttaaggtagccttgcagaagttggtcgtgaggcactgggcaggtaagtatcaaggttacaagacaggtttaaggagaccaatagaaactgggcttgtcgagacagagaaaaacctaacccccatggttggcgagggactgctgtgtgtgaaatggtaactgccctcaaggagcttacaatctagctgggggtaaatgacttgcacatgaacacaactagactgtgagcttctagagggcagggaccttaccctagtcatctctcttctcaccctgcacaccctccctgagggatctcatgactcttgcgtttctgataggcacctattggtcttactgacatccactttgcctttctctccacaggtgtccactcccagttcacaccggcacaatgaatggcacagaaggccctaacttctacgtgcccttctccaatgcgacgggtgtggtacgcagccccttcgagtacccacagtcagagataaatgacagtgacagcaacgtgagctgcagcccttaggactgagaaagcatcgagaccaggggtctccggcaaggcctaggtcctcccttcagtatggaaaccttgcctcatgtctctcagcctccttggcctgtggagatccagcccttcctcttggcttctggatacatttgctcttctacaccagcaaccaagtggcaacagttccaggccagtatggagttttagaagccatgccaatatgcccaccttcagggagcagctgagtccttgatgccacccttgttctgaagagttcagaaacacagtgcaagacatgaccaggcctcatccttaggatgctcatggatccagttcttagctcccttgttggatatgctgttttccttggcctttggtcttttctttatcccagagggttttggctttaaggccaacaggaactatggggtaccagaattgagcagcctcagtctgcatccctcctctatagaaccacagctgggccctcagcaggcccaactctgcatggggacagaggcattaaaagc

SEQ ID NO: 8 - DNA, 1826 bp, Artificial Sequence
  Synthetic Construct
gggccccagaagcctggtggttgtttgtccttctcaggggaaaagtgaggcggccccttggaggaaggggccgggcagaatgatctaatcggattccaagcagctcaggggattgtctttttctagcaccttcttgccactcctaagcgtcctccgtgaccccggctgggatttagcctggtgctgtgtcagccccggtctcccaggggcttcccagtggtccccaggaaccctcgacagggcccggtctctctcgtccagcaagggcagggacgggccacaggccaagggcactagaagctttattgcggtagtttatcacagttaaattgctaacgcagtcagtgcttctgacacaacagtctcgaacttaagctgcagtgactctcttaaggtagccttgcagaagttggtcgtgaggcactgggcaggtaagtatcaaggttacaagacaggtttaaggagaccaatagaaactgggcttgtcgagacagagaaaaacctaacccccatggttggcgagggactgctgtgtgtgaaatggtaactgccctcaaggagcttacaatctagctgggggtaaatgacttgcacatgaacacaactagactgtgagcttctagagggcagggaccttaccctagtcatctctcttctcaccctgcacaccctccctgagggatctcatgactcttgcgtttctgataggcacctattggtcttactgacatccactttgcctttctctccacaggtgtccactcccagttcacaccggcacaatgaatggcacagaaggccctaacttctacgtgcccttctccaatgcgacgggtgtggtacgcagccccttcgagtacccacagtactacctggctgagccatggcagttctccatgctggccgcctacatgtttctgctgatcgtgctgggcttccccatcaacttcctcacgctctacgtcaccgtccagcacaagaagctgcgcacgcctctcaactacatcctgctcaacctagccgtggctgacctcttcatggtcctaggtggcttcaccagcaccctctacacctctctgcatggatacttcgtcttcgggcccacaggatgcaatttggagggcttctttgccaccctgggcggtgaaattgccctgtggtccttggtggtcctggccatcgagcggtacgtggtggtgtgtaagcccatgagcaacttccgcttcggggagaaccatgccatcatgggcgttgccttcacctgggtcatggcgctggcctgcgccgcacccccactcgccggctggtccaggtacatccccgagggcctgcagtgctcgtgtggaatcgactactacacgctcaagccggaggtcaacaacgagtcttttgtcatctacatgttcgtggtccacttcaccatccccatgattatcatctttttctgctatgggcagctcgtcttcaccgtcaaggaggccgctgcccagcagcaggagtcagccaccacacagaaggcagagaaggaggtcacccgcatggtcatcatcatggtcatcgctttcctgatctgctgggtgccctacgccagcgtggcattctacatcttcacccaccagggctccaacttcggtcccatcttcatgaccatcccagcgttctttgccaagagcgccgccatctacaaccctgtcatctatatcatgatgaacaagcagttccggaactgcatgctcaccaccatctgctgcggcaagaacccactgggtgacgatgaggcctctgctaccgtgtccaagacggagacgagccaggtggccccggcc

SEQ ID NO: 9 - DNA, 3444 bp, Artificial Sequence; identical to SEQ ID NO: 6
  Synthetic Construct

SEQ ID NO: 10 - DNA, 1017 bp, Artificial Sequence
  Synthetic Construct
ggagtcgctgcgacgctgccttcgccccgtgccccgctccgccgccgcctcgcgccgcccgccccggctctgactgaccgcgttactcccacaggtgagcgggcgggacggcccttctcctccgggctgtaattagcgcttggtttaatgacggcttgtttcttttctgtggctgcgtgaaagccttgaggggctccgggagggccctttgtgcggggggagcggctcggggggtgcgtgcgtgtgtgtgtgcgtggggagcgccgcgtgcggctccgcgctgcccggcggctgtgagcgctgcgggcgcggcgcggggctttgtgcgctccgcagtgtgcgcgaggggagcgcggccgggggcggtgccccgcggtgcggggggggctgcgaggggaacaaaggctgcgtgcggggtgtgtgcgtgggggggtgagcagggggtgtgggcgcgtcggtcgggctgcaaccccccctgcacccccctccccgagttgctgagcacggcccggcttcgggtgcggggctccgtacggggcgtggcgcggggctcgccgtgccgggcggggggtggcggcaggtgggggtgccgggcggggcggggccgcctcgggccggggagggctcgggggaggggcgcggcggcccccggagcgccggcggctgtcgaggcgcggcgagccgcagccattgccttttatggtaatcgtgcgagagggcgcagggacttcctttgtcccaaatctgtgcggagccgaaatctgggaggcgccgccgcaccccctctagcgggcgcggggcgaagcggtgcggcgccggcaggaaggaaatgggcggggagggccttcgtgcgtcgccgcgccgccgtccccttctccctctccagcctcggggctgtccgcggggggacggctgccttcgggggggacggggcagggcggggttcggcttctggcgtgtgaccggcggctctagagcctctgctaaccatgttcatgccttcttctttttcctaca

SEQ ID NO: 11 - DNA, 2239 bp, Artificial Sequence
  Synthetic Construct
aagcttgaaatgccacctcctctgatattctaggtgtcctggaagcctgtctcatcttgccctgtagtgttgggtcacctggcccccagcctgtaacatccccagggccctacacccagagaaacacggggctggtggcagtgcccagtgacaaccgtttagtggataagagaagagtgaccacaccaggctgagtgctcctctctggttttccatggggagacaatgccaccctgagcagggtctggtgtgagcggcagctggctctgggctctctgatccgttaccctctcagcctctttgttctttctcaacccctggagcagagacctcaggaggtgctggcatggaacagagaaattccagcctcgattcctattatgaacccgacaccttttgtattttcatcttggttttacagtgtacaaaacgaactagatcagcagggcatgggcataatcacgaatgcacacacatacactaatgtgtggctcatgtttaagtatcacttactacaggacacccaatctaacagcaccgataaagtgacagagaaacgcaagccttctgcgaacatggcctggctgttccaattccgaaccttgcttttctgggccttgccacacaggctcttcccccgtccccccagggacattctacccttgaactccacactccactgctgcctttgccaggaagcccatctgttcctttttggttctgccagaacgtgtggtggtgctgctgtccctgccttgggcactggatattgggaagggacagtgtccacactggagtgggaagttcccagggacgagacctttacctcctcaccctgggtactgttctcctcatggagcatggacggcgctgcctgaactcagtggtggcctcattctggaagccaagtttatacagagtagcagtgacccagggatgtggggttcaccctcctcagccctctggccagtcctgatgggcctcagtcccaacatggctaagaggtgtgggcagcttcttggtcaccctcaggttggggaatcaccttctgtcttcattttccaggaacttggtgatgatatcgtgggtgagttcatttaccaggtgctgtagtttcccctcatcaggcaggaagaagatggcggtggcattgcccaggtatttcatcagcagcacccagctggacagcttcttacagtgctggatgttaaacatgcctaaacgcttcatcataggcaccttcacggtggtcacctggtccacgtggaagtcctcttcctcggtgtccttgacttcaaagggtctctcccatttgcctggagagaggggaaggtgggcatcaccaggggtgagtgaaggtttggaagagtgtagcagaataagaaaccatgagtcccctccctgagaagccctgagcccccttgacgacacacatccctcgaggctcagcttcatcatctgtaaaaggtgctgaaactgaccatccaagctgccgaaaaagattgtgtggggataattcaaaactagaggaagatgcagaatttctacatcgtggcgatgtcaggctaagagatgccatcgtggctgtgcatttttattggaatcatatgtttatttgagggtgtcttggatattacaaataaaatgttggagcatcaggcatatttggtaccttctgtctaaggctccctgccccttgttaattggcagctcagttattcatccagggcaaacattctgcttactattcctgagagctttcctcatcctctagattggcaggggaaatgcagatgcctgagcagcctcccctctgccataccaacagagcttcaccatcgaggcatgcagagtggacaggggcctcagggacccctgatcccagctttctcattggacagaaggaggagactggggctggagagggacctgggcccccactaaggccacagcagagccaggactttagctgtgctgactgcagcctggcttgcctccactgccctcctttgcctcaagagcaagggagcctcagagtggaggaagcagcccctggccttgcctcccacctcccctcccctatgctgttttcctgggacagtgggagctggcttagaatgccctggggcccccaggaccctggcattttaacccctcaggggcaggaaggcagcctgagatacagaagagtccatcacctgctgtatgccacacaccatccccacagttacgtactagt

SEQ ID NO: 12 - DNA, 6408 bp, Artificial Sequence
  Synthetic Construct
gaattcggaccgtcgacattgattattgactagttattaatagtaatcaattacggggtcattagttcatagcccatatatggagttccgcgttacataacttacggtaaatggcccgcctggctgaccgcccaacgacccccgcccattgacgtcaataatgacgtatgttcccatagtaacgccaatagggactttccattgacgtcaatgggtggagtatttacggtaaactgcccacttggcagtacatcaagtgtatcatatgccaagtacgccccctattgacgtcaatgacggtaaatggcccgcctggcattatgcccagtacatgaccttatgggactttcctacttggcagtacatctacgtattagtcatcgctattaccatggtcgaggtgagccccacgttctgcttcactctccccatctcccccccctccccacccccaattttgtatttatttattttttaattattttgtgcagcgatgggggcggggggggggggggggcgcgcgccaggcggggcggggcggggcgaggggcggggcggggcgaggcggagaggtgcggcggcagccaatcagagcggcgcgctccgaaagtttccttttatggcgaggcggcggcggcggcggccctataaaaagcgaagcgcgcggcgggcggggagtcgctgcgacgctgccttcgccccgtgccccgctccgccgccgcctcgcgccgcccgccccggctctgactgaccgcgttactcccacaggtgagcgggcgggacggcccttctcctccgggctgtaattagcgcttggtttaatgacggcttgtttcttttctgtggctgcgtgaaagccttgaggggctccgggagggccctttgtgcggggggagcggctcggggggtgcgtgcgtgtgtgtgtgcgtggggagcgccgcgtgcggctccgcgctgcccggcggctgtgagcgctgcgggcgcggcgcggggctttgtgcgctccgcagtgtgcgcgaggggagcgcggccgggggcggtgccccgcggtgcggggggggctgcgaggggaacaaaggctgcgtgcggggtgtgtgcgtgggggggtgagcagggggtgtgggcgcgtcggtcgggctgcaaccccccctgcacccccctccccgagttgctgagcacggcccggcttcgggtgcggggctccgtacggggcgtggcgcggggctcgccgtgccgggcggggggtggcggcaggtgggggtgccgggcggggcggggccgcctcgggccggggagggctcgggggaggggcgcggcggcccccggagcgccggcggctgtcgaggcgcggcgagccgcagccattgccttttatggtaatcgtgcgagagggcgcagggacttcctttgtcccaaatctgtgcggagccgaaatctgggaggcgccgccgcaccccctctagcgggcgcggggcgaagcggtgcggcgccggcaggaaggaaatgggcggggagggccttcgtgcgtcgccgcgccgccgtccccttctccctctccagcctcggggctgtccgcggggggacggctgccttcgggggggacggggcagggcggggttcggcttctggcgtgtgaccggcggctctagagcctctgctaaccatgttcatgccttcttctttttcctacagctcctgggcaacgtgctggttattgtgctgtctcatcattttggcaaagaattcttcgaaagatctgctagcttaattaacccaaacgggccctctagactcgagcggccgccactgtgctggatatctgcagaattcagccaccaccggcacaatgaatggcacagaaggccctaacttctacgtgcccttctccaatgcgacgggtgtggtacgcagccccttcgagtacccacagtactacctggctgagccatggcagttctccatgctggccgcctacatgtttctgctgatcgtgctgggcttccccatcaacttcctcacgctctacgtcaccgtccagcacaagaagctgcgcacgcctctcaactacatcctgctcaacctagccgtggctgacctcttcatggtcctaggtggcttcaccagcaccctctacacctctctgcatggatacttcgtcttcgggcccacaggatgcaatttggagggcttctttgccaccctgggcggtgaaattgccctgtggtccttggtggtcctggccatcgagcggtacgtggtggtgtgtaagcccatgagcaacttccgcttcggggagaaccatgccatcatgggcgttgccttcacctgggtcatggcgctggcctgcgccgcacccccactcgccggctggtccaggtacatccccgagggcctgcagtgctcgtgtggaatcgactactacacgctcaagccggaggtcaacaacgagtcttttgtcatctacatgttcgtggtccacttcaccatccccatgattatcatctttttctgctatgggcagctcgtcttcaccgtcaaggaggccgctgcccagcagcaggagtcagccaccacacagaaggcagagaaggaggtcacccgcatggtcatcatcatggtcatcgctttcctgatctgctgggtgccctacgccagcgtggcattctacatcttcacccaccagggctccaacttcggtcccatcttcatgaccatcccagcgttctttgccaagagcgccgccatctacaaccctgtcatctatatcatgatgaacaagcagttccggaactgcatgctcaccaccatctgctgcggcaagaacccactgggtgacgatgaggcctctgctaccgtgtccaagacggagacgagccaggtggccccggcctaaccaagaaagcttaagtttgggactagtggcggccgctcgagcatgcatctagagggccctattctatagtgtcacctaaatgctagagctcgctgatcagcctcgactgtgccttctagttgccagccatctgttgtttgcccctcccccgtgccttccttgaccctggaaggtgccactcccactgtcctttcctaataaaatgaggaaattgcatcgcattgtctgagtaggtgtcattctattctggggggtggggtggggcaggacagcaagggggaggattgggaagacaatagcaggcatgctggggagctagagtcgaccggaccgctgcaggcatgcaagcttggcgtaatcatggtcatagctgtttcctgtgtgaaattgttatccgctcacaattccacacaacatacgagccggaagcataaagtgtaaagcctggggtgcctaatgagtgagctaactcacattaattgcgttgcgctcactgcccgctttccagtcgggaaacctgtcgtgccagctgcattaatgaatcggccaacgcgcggggagaggcggtttgcgtattgggcgctcttccgtattagtcatcgctattaccatggtgatgcggttttggcagtacatcaatgggcgtggatagcggtttgactcacggggatttccaagtctccaccccattgacgtcaatgggagtttgttttggcaccaaaatcaacgggactttccaaaatgtcgtaacaactccgccccattgacgcaaatgggcggtaggcgtgtacggtgggaggtctatataagcagagctctctggctaactagagaacccactgcttactggcttatcgaaattaatacgactcactatagggagtcccaagctggctagttaagctatcaacaagtttgtacaaaaaagcaggctttaaagggaggtagtgagtcgaccagtggatcctggaggcttgctgaaggctgtatgctgaaggagcttacaatctagctggggttttggccactgactgaccccagctagtgtaagctccttcaggacacaaggcctgttactagcactcacatggaacaaatggcccagatctggccgcactcgagatgcttcctcgctcactgactcgctgcgctcggtcgttcggctgcggcgagcggtatcagctcactcaaaggcggtaatacggttatccacagaatcaggggataacgcaggaaagaacatgtgagcaaaaggccagcaaaaggccaggaaccgtaaaaaggccgcgttgctggcgtttttccataggctccgcccccctgacgagcatcacaaaaatcgacgctcaagtcagaggtggcgaaacccgacaggactataaagataccaggcgtttccccctggaagctccctcgtgcgctctcctgttccgaccctgccgcttaccggatacctgtccgcctttctcccttcgggaagcgtggcgctttctcatagctcacgctgtaggtatctcagttcggtgtaggtcgttcgctccaagctgggctgtgtgcacgaaccccccgttcagcccgaccgctgcgccttatccggtaactatcgtcttgagtccaacccggtaagacacgacttatcgccactggcagcagccactggtaacaggattagcagagcgaggtatgtaggcggtgctacagagttcttgaagtggtggcctaactacggctacactagaaggacagtatttggtatctgcgctctgctgaagccagttaccttcggaaaaagagttggtagctcttgatccggcaaacaaaccaccgctggtagcggtggtttttttgtttgcaagcagcagattacgcgcagaaaaaaaggatctcaagaagatcctttgatcttttctacggggtctgacgctcagtggaacgaaaactcacgttaagggattttggtcatgagattatcaaaaaggatcttcacctagatccttttaaattaaaaatgaagttttaaatcaatctaaagtatatatgagtaaacttggtctgacagttaccaatgcttaatcagtgaggcacctatctcagcgatctgtctatttcgttcatccatagttgcctgactccccgtcgtgtagataactacgatacgggagggcttaccatctggccccagtgctgcaatgataccgcgagacccacgctcaccggctccagatttatcagcaataaaccagccagccggaagggccgagcgcagaagtggtcctgcaactttatccgcctccatccagtctattaattgttgccgggaagctagagtaagtagttcgccagttaatagtttgcgcaacgttgttgccattgctacaggcatcgtggtgtcacgctcgtcgtttggtatggcttcattcagctccggttcccaacgatcaaggcgagttacatgatcccccatgttgtgcaaaaaagcggttagctccttcggtcctccgatcgttgtcagaagtaagttggccgcagtgttatcactcatggttatggcagcactgcataattctcttactgtcatgccatccgtaagatgcttttctgtgactggtgagtactcaaccaagtcattctgagaatagtgtatgcggcgaccgagttgctcttgcccggcgtcaatacgggataataccgcgccacatagcagaactttaaaagtgctcatcattggaaaacgttcttcggggcgaaaactctcaaggatcttaccgctgttgagatccagttcgatgtaacccactcgtgcacccaactgatcttcagcatcttttactttcaccagcgtttctgggtgagcaaaaacaggaaggcaaaatgccgcaaaaaagggaataagggcgacacggaaatgttgaatactcatactcttcctttttcaatattattgaagcatttatcagggttattgtctcatgagcggatacatatttgaatgtatttagaaaaataaacaaataggggttccgcgcacatttccccgaaaagtgccacctgacgtctaagaaaccattattatcatgacattaacctataaaaataggcgtatcacgaggccctttcgtctcgcgcgtttcggtgatgacggtgaaaacctctgacacatgcagctcccggagacggtcacagcttgtctgtaagcggatgccgggagcagacaagcccgtcagggcgcgtcagcgggtgttggcgggtgtcggggctggcttaactatgcggcatcagagcagattgtactgagagtgcaccatatgcggtgtgaaataccgcacagatgcgtaaggagaaaataccgcatcaggcgccattcgccattcaggctgcgcaactgttgggaagggcgatcggtgcgggcctcttcgctattacgccagctggcgaaagggggatgtgctgcaaggcgattaagttgggtaacgccagggttttcccagtcacgacgttgtaaaacgacggccagt

SEQ ID NO: 13 - DNA, 155 bp, Artificial Sequence
  Synthetic Construct
gatcctggaggcttgctgaaggctgtatgctgaaggagcttacaatctagctggggttttggccactgactgaccccagctagtgtaagctccttcaggacacaaggcctgttactagcactcacatggaacaaatggcccagatctggccgcac

SEQ ID NO: 14 - DNA, 189 bp, Homo sapiens
aacctaacccccatggttggcgagggactgctgtgtgtgaaatggtaactgccctcaaggagcttacaatctagctgggggtaaatgacttgcacatgaacacaactagactgtgagcttctagagggcagggaccttaccctagtcatctctcttctcaccctgcacaccctccctgagggatctcat

SEQ ID NO: 15 - DNA, 6172 bp, Artificial Sequence
  Synthetic Construct
tatgcggtgtgaaataccgcacagatgcgtaaggagaaaataccgcatcaggcgccattcgccattcaggctgcgcaactgttgggaagggcgatcggtgcgggcctcttcgctattacgccagctggcgaaagggggatgtgctgcaaggcgattaagttgggtaacgccagggttttcccagtcacgacgttgtaaaacgacggccagtgaattcggaccgtcgacattgattattgggccccagaagcctggtggttgtttgtccttctcaggggaaaagtgaggcggccccttggaggaaggggccgggcagaatgatctaatcggattccaagcagctcaggggattgtctttttctagcaccttcttgccactcctaagcgtcctccgtgaccccggctgggatttagcctggtgctgtgtcagccccggtctcccaggggcttcccagtggtccccaggaaccctcgacagggcccggtctctctcgtccagcaagggcagggacgggccacaggccaagggcggagtcgctgcgacgctgccttcgccccgtgccccgctccgccgccgcctcgcgccgcccgccccggctctgactgaccgcgttactcccacaggtgagcgggcgggacggcccttctcctccgggctgtaattagcaagaggtaagggtttaagggatggttggttggtggggtattaatgtttaattacctgttttacaggcctgaaatcacttggttttaggttggggatccggtacccaattgccatgggctagcatgcatgagctccctgcagggtttatctgcagaattcagccaccaccggcacaatgaatggcacagaaggccctaacttctacgtgcccttctccaatgcgacgggtgtggtacgcagccccttcgagtacccacagtactacctggctgagccatggcagttctccatgctggccgcctacatgtttctgctgatcgtgctgggcttccccatcaacttcctcacgctctacgtcaccgtccagcacaagaagctgcgcacgcctctcaactacatcctgctcaacctagccgtggctgacctcttcatggtcctaggtggcttcaccagcaccctctacacctctctgcatggatacttcgtcttcgggcccacaggatgcaatttggagggcttctttgccaccctgggcggtgaaattgccctgtggtccttggtggtcctggccatcgagcggtacgtggtggtgtgtaagcccatgagcaacttccgcttcggggagaaccatgccatcatgggcgttgccttcacctgggtcatggcgctggcctgcgccgcacccccactcgccggctggtccaggtacatccccgagggcctgcagtgctcgtgtggaatcgactactacacgctcaagccggaggtcaacaacgagtcttttgtcatctacatgttcgtggtccacttcaccatccccatgattatcatctttttctgctatgggcagctcgtcttcaccgtcaaggaggccgctgcccagcagcaggagtcagccaccacacagaaggcagagaaggaggtcacccgcatggtcatcatcatggtcatcgctttcctgatctgctgggtgccctacgccagcgtggcattctacatcttcacccaccagggctccaacttcggtcccatcttcatgaccatcccagcgttctttgccaagagcgccgccatctacaaccctgtcatctatatcatgatgaacaagcagttccggaactgcatgctcaccaccatctgctgcggcaagaacccactgggtgacgatgaggcctctgctaccgtgtccaagacggagacgagccaggtggccccggcctaaccaagaaagcttaagtttgtgtcccggcttagggctaaatgtctaggacagaatggaacacatagtagctgattaataaatgctagctggatgaagggaggaatgagtgactgactgagtggatatatgagtgaagggattaatggaagggaacatggatgtcctcaggtgcccaacctggcagatccagtcatgtctggctggaatctataagcagttttacatacctgccctgagctttattgcggtagtttatcacagttaaattgctaacgcagtcagtgcttctgacacaacagtctcgaacttaagctgcagtgactctcttaaggtagccttgcagaagttggtcgtgaggcactgggcaggtaagtatcaaggttacaagacaggtttaaggagaccaatagaaactgggcttgtcgagacagagaaaaacctaacccccatggttggcgagggactgctgtgtgtgaaatggtaactgccctcaaggagcttacaatctagctgggggtaaatgacttgcacatgaacacaactagactgtgagcttctagagggcagggaccttaccctagtcatctctcttctcaccctgcacaccctccctgagggatctcatgactcttgcgtttctgataggcacctattggtcttactgacatccactttgcctttctctccacaggtgtccactcccagttcacaccggcacaatgaatggcacagaaggccctaacttctacgtgcccttctccaatgcgacgggtgtggtacgcagccccttcgagtacccacagtcagagataaatgacagtgacagcaacgtgagctgcagcccttaggactgagaaagcatcgagaccaggggtctccggcaaggcctaggtcctcccttcagtatggaaaccttgcctcatgtctctcagcctccttggcctgtggagatccagcccttcctcttggcttctggatacatttgctcttctacaccagcaaccaagtggcaacagttccaggccagtatggagttttagaagccatgccaatatgcccaccttcagggagcagctgagtccttgatgccacccttgttctgaagagttcagaaacacagtgcaagacatgaccaggcctcatccttaggatgctcatggatccagttcttagctcccttgttggatatgctgttttccttggcctttggtcttttctttatcccagagggttttggctttaaggccaacaggaactatggggtaccagaattgagcagcctcagtctgcatccctcctctatagaaccacagctgggccctcagcaggcccaactctgcatggggacagaggcattaaaagcctagagtatccctcgaggggcccaagcttacgcgtacccagctttcttgtacaaagtggtccctatagtgagtcgtattataagctaggcactggccgtcgttttacaacgtcgtgactgggaaaactgctagcttgggatctttgtgaaggaaccttacttctgtggtgtgacataattggacaaactacctacagagatttaaagctctaaggtaaatataaaatttttaagtgtataatgtgttaaactagctgcaaaacctgtgccttctagttgccagccatctgttgtttgcccctcccccgtgccttccttgaccctggaaggtgccactcccactgtcctttcctaataaaatgaggaaattgcatcgcattgtctgagtaggtgtcattctattctggggggtggggtggggcaggacagcaagggggaggattgggaagacaatagcaggcatgctggggaactagtcggaccgctgcaggcatgcaagcttggcgtaatcatggtcatagctgtttcctgtgtgaaattgttatccgctcacaattccacacaacatacgagccggaagcataaagtgtaaagcctggggtgcctaatgagtgagctaactcacattaattgcgttgcgctcactgcccgctttccagtcgggaaacctgtcgtgccagctgcattaatgaatcggccaacgcgcggggagaggcggtttgcgtattgggcgctcttccgcttcctcgctcactgactcgctgcgctcggtcgttcggctgcggcgagcggtatcagctcactcaaaggcggtaatacggttatccacagaatcaggggataacgcaggaaagaacatgtgagcaaaaggccagcaaaaggccaggaaccgtaaaaaggccgcgttgctggcgtttttccataggctccgcccccctgacgagcatcacaaaaatcgacgctcaagtcagaggtggcgaaacccgacaggactataaagataccaggcgtttccccctggaagctccctcgtgcgctctcctgttccgaccctgccgcttaccggatacctgtccgcctttctcccttcgggaagcgtggcgctttctcatagctcacgctgtaggtatctcagttcggtgtaggtcgttcgctccaagctgggctgtgtgcacgaaccccccgttcagcccgaccgctgcgccttatccggtaactatcgtcttgagtccaacccggtaagacacgacttatcgccactggcagcagccactggtaacaggattagcagagcgaggtatgtaggcggtgctacagagttcttgaagtggtggcctaactacggctacactagaaggacagtatttggtatctgcgctctgctgaagccagttaccttcggaaaaagagttggtagctcttgatccggcaaacaaaccaccgctggtagcggtggtttttttgtttgcaagcagcagattacgcgcagaaaaaaaggatctcaagaagatcctttgatcttttctacggggtctgacgctcagtggaacgaaaactcacgttaagggattttggtcatgagattatcaaaaaggatcttcacctagatccttttaaattaaaaatgaagttttaaatcaatctaaagtatatatgagtaaacttggtctgacagttaccaatgcttaatcagtgaggcacctatctcagcgatctgtctatttcgttcatccatagttgcctgactccccgtcgtgtagataactacgatacgggagggcttaccatctggccccagtgctgcaatgataccgcgagacccacgctcaccggctccagatttatcagcaataaaccagccagccggaagggccgagcgcagaagtggtcctgcaactttatccgcctccatccagtctattaattgttgccgggaagctagagtaagtagttcgccagttaatagtttgcgcaacgttgttgccattgctacaggcatcgtggtgtcacgctcgtcgtttggtatggcttcattcagctccggttcccaacgatcaaggcgagttacatgatcccccatgttgtgcaaaaaagcggttagctccttcggtcctccgatcgttgtcagaagtaagttggccgcagtgttatcactcatggttatggcagcactgcataattctcttactgtcatgccatccgtaagatgcttttctgtgactggtgagtactcaaccaagtcattctgagaatagtgtatgcggcgaccgagttgctcttgcccggcgtcaatacgggataataccgcgccacatagcagaactttaaaagtgctcatcattggaaaacgttcttcggggcgaaaactctcaaggatcttaccgctgttgagatccagttcgatgtaacccactcgtgcacccaactgatcttcagcatcttttactttcaccagcgtttctgggtgagcaaaaacaggaaggcaaaatgccgcaaaaaagggaataagggcgacacggaaatgttgaatactcatactcttcctttttcaatattattgaagcatttatcagggttattgtctcatgagcggatacatatttgaatgtatttagaaaaataaacaaataggggttccgcgcacatttccccgaaaagtgccacctgacgtctaagaaaccattattatcatgacattaacctataaaaataggcgtatcacgaggccctttcgtctcgcgcgtttcggtgatgacggtgaaaacctctgacacatgcagctcccggagacggtcacagcttgtctgtaagcggatgccgggagcagacaagcccgtcagggcgcgtcagcgggtgttggcgggtgtcggggctggcttaactatgcggcatcagagcagattgtactgagagtgcacca

SEQ ID NO: 16 - DNA, 441 bp, Homo sapiens
actagaagctttattgcggtagtttatcacagttaaattgctaacgcagtcagtgcttctgacacaacagtctcgaacttaagctgcagtgactctcttaaggtagccttgcagaagttggtcgtgaggcactgggcaggtaagtatcaaggttacaagacaggtttaaggagaccaatagaaactgggcttgtcgagacagagaatggatcctggaggcttgctgaaggctgtatgctgaaggagcttacaatctagctggggttttggccactgactgaccccagctagtgtaagctccttcaggacacaaggcctgttactagcactcacatggaacaaatggcccagatctgagactcttgcgtttctgataggcacctattggtcttactgacatccactttgcctttctctccacaggtgtccactcccagttca

SEQ ID NO: 17 - DNA, 150 bp, Artificial Sequence
  Synthetic Construct
tggatcctggaggcttgctgaaggctgtatgctgaaggagcttacaatctagctggggttttggccactgactgaccccagctagtgtaagctccttcaggacacaaggcctgttactagcactcacatggaacaaatggcccagatctg

SEQ ID NO: 18 - DNA, 190 bp, Homo sapiens
aaacctaacccccatggttggcgagggactgctgtgtgtgaaatggtaactgccctcaaggagcttacaatctagctgggggtaaatgacttgcacatgaacacaactagactgtgagcttctagagggcagggaccttaccctagtcatctctcttctcaccctgcacaccctccctgagggatctcat

SEQ ID NO: 19 - RNA, 79 nt, Homo sapiens
cucugccuggagacuaaggcaaauugggccauuaaaagcucagcuccuauguugguauuaacggugguggguuuuguug

SEQ ID NO: 20 - DNA, 113 bp, Artificial Sequence
  Synthetic Construct
ccactccctctctgcgcgctcgctcgctcactgaggccgggcgaccaaaggtcgcccgacgcccgggctttgcccgggcggcctcagtgagcgagcgagcgcgcagagaggga

SEQ ID NO: 21 - DNA, 143 bp, Artificial Sequence
  Synthetic Construct
ggccactccctctctgcgcgctcgctcgctcactgaggccgggcgaccaaaggtcgcccgacgcccgggctttgcccgggcggcctcagtgagcgagcgagcgcgcagagagggagtggccaactccatcactaggggttcct

SEQ ID NO: 22 - DNA, 795 bp, Mus musculus
tgctgattcagccaggaactagttattaatagtaatcaattacggggtcattagttcatagcccatatatggagttccgcgttacataacttacggtaaatggcccgcctggctgaccgcccaacgacccccgcccattgacgtcaataatgacgtatgttcccatagtaacgccaatagggactttccattgacgtcaatgggtggagtatttacggtaaactgcccacttggcagtacatcaagtgtatcatatgccaagtacgccccctattgacgtcaatgacggtaaatggcccgcctggcattatgcccagtacatgaccttatgggactttcctacttggcagtacatctacgtattagtcatcgctattaccacaaatagttatcgagccgctgagccggggggcggggggtgtgagactggaggcgatggacggagctgacggcacacacagctcagatctgtcaagtgagccattgtcagggcttggggactggataagtcagggggtctcctgggaagagatgggataggtgagttcaggaggagacattgtcaactggagccatgtggagaagtgaatttagggcccaaaggttccagtcgcagcctgaggccaccagactgacatggggaggaattcccagaggactctggggcagacaagatgagacaccctttcctttctttacctaagggcctccacccgatgtcaccttggcccctctgcaagccaattaggccccggtggcagcagtgggattagcgttagtatgatatctcgcgga

SEQ ID NO: 23 - DNA, 315 bp, Artificial Sequence
  Synthetic Construct
ggagtcgctgcgacgctgccttcgccccgtgccccgctccgccgccgcctcgcgccgcccgccccggctctgactgaccgcgttactcccacaggtgagcgggcgggacggcccttctcctccgggctgtaattagcaagaggtaagggtttaagggatggttggttggtggggtattaatgtttaattacctgttttacaggcctgaaatcacttggttttaggttggggatccggtacccaattgccatgggctagcatgcatgagctccctgcagggttttaatgccaactttgtacaaaaaagcaggcacc

SEQ ID NO: 24 - DNA, 2064 bp, Artificial Sequence
  Synthetic Construct
tgactagttagggccccagaagcctggtggttgtttgtccttctcaggggaaaagtgaggcggccccttggaggaaggggccgggcagaatgatctaatcggattccaagcagctcaggggattgtctttttctagcaccttcttgccactcctaagcgtcctccgtgaccccggctgggatttagcctggtgctgtgtcagccccggtctcccaggggcttcccagtggtccccaggaaccctcgacagggcccggtctctctcgtccagcaagggcagggacgggccacaggccaagggcactagaagctttattgcggtagtttatcacagttaaattgctaacgcagtcagtgcttctgacacaacagtctcgaacttaagctgcagtgactctcttaaggtagccttgcagaagttggtcgtgaggcactgggcaggtaagtatcaaggttacaagacaggtttaaggagaccaatagaaactgggcttgtcgagacagagaatggatcctggaggcttgctgaaggctgtatgctgaaggagcttacaatctagctggggttttggccactgactgaccccagctagtgtaagctccttcaggacacaaggcctgttactagcactcacatggaacaaatggcccagatctgagactcttgcgtttctgataggcacctattggtcttactgacatccactttgcctttctctccacaggtgtccactcccagttcacaccggcacaatgaatggcacagaaggccctaacttctacgtgcccttctccaatgcgacgggtgtggtacgcagccccttcgagtacccacagtactacctggctgagccatggcagttctccatgctggccgcctacatgtttctgctgatcgtgctgggcttccccatcaacttcctcacgctctacgtcaccgtccagcacaagaagctgcgcacgcctctcaactacatcctgctcaacctagccgtggctgacctcttcatggtcctaggtggcttcaccagcaccctctacacctctctgcatggatacttcgtcttcgggcccacaggatgcaatttggagggcttctttgccaccctgggcggtgaaattgccctgtggtccttggtggtcctggccatcgagcggtacgtggtggtgtgtaagcccatgagcaacttccgcttcggggagaaccatgccatcatgggcgttgccttcacctgggtcatggcgctggcctgcgccgcacccccactcgccggctggtccaggtacatccccgagggcctgcagtgctcgtgtggaatcgactactacacgctcaagccggaggtcaacaacgagtcttttgtcatctacatgttcgtggtccacttcaccatccccatgattatcatctttttctgctatgggcagctcgtcttcaccgtcaaggaggccgctgcccagcagcaggagtcagccaccacacagaaggcagagaaggaggtcacccgcatggtcatcatcatggtcatcgctttcctgatctgctgggtgccctacgccagcgtggcattctacatcttcacccaccagggctccaacttcggtcccatcttcatgaccatcccagcgttctttgccaagagcgccgccatctacaaccctgtcatctatatcatgatgaacaagcagttccggaactgcatgctcaccaccatctgctgcggcaagaacccactgggtgacgatgaggcctctgctaccgtgtccaagacggagacgagccaggtggccccggcctaaccaagaaagcttaagtttaaaccgctgatcagcctcgactgtgccttctagttgccagccatctgttgtttgcccctcccccgtgccttccttgaccctggaaggtgccactcccactgtcctttcctaataaaatgaggaaattgcatcgcattgtctgagtaggtgtcattctattctggggggtggggtggggcaggacagcaagggggaggattgggaagacaatagcaggcatgctggggatgcggtgggctctatggc

SEQ ID NO: 25 - DNA, 2093 bp, Artificial Sequence
  Synthetic Construct
gggccccagaagcctggtggttgtttgtccttctcaggggaaaagtgaggcggccccttggaggaaggggccgggcagaatgatctaatcggattccaagcagctcaggggattgtctttttctagcaccttcttgccactcctaagcgtcctccgtgaccccggctgggatttagcctggtgctgtgtcagccccggtctcccaggggcttcccagtggtccccaggaaccctcgacagggcccggtctctctcgtccagcaagggcagggacgggccacaggccaagggcactagaagctttattgcggtagtttatcacagttaaattgctaacgcagtcagtgcttctgacacaacagtctcgaacttaagctgcagtgactctcttaaggtagccttgcagaagttggtcgtgaggcactgggcaggtaagtatcaaggttacaagacaggtttaaggagaccaatagaaactgggcttgtcgagacagagaaaaacctaacccccatggttggcgagggactgctgtgtgtgaaatggtaactgccctcaaggagcttacaatctagctgggggtaaatgacttgcacatgaacacaactagactgtgagcttctagagggcagggaccttaccctagtcatctctcttctcaccctgcacaccctccctgagggatctcatgactcttgcgtttctgataggcacctattggtcttactgacatccactttgcctttctctccacaggtgtccactcccagttcacaccggcacaatgaatggcacagaaggccctaacttctacgtgcccttctccaatgcgacgggtgtggtacgcagccccttcgagtacccacagtactacctggctgagccatggcagttctccatgctggccgcctacatgtttctgctgatcgtgctgggcttccccatcaacttcctcacgctctacgtcaccgtccagcacaagaagctgcgcacgcctctcaactacatcctgctcaacctagccgtggctgacctcttcatggtcctaggtggcttcaccagcaccctctacacctctctgcatggatacttcgtcttcgggcccacaggatgcaatttggagggcttctttgccaccctgggcggtgaaattgccctgtggtccttggtggtcctggccatcgagcggtacgtggtggtgtgtaagcccatgagcaacttccgcttcggggagaaccatgccatcatgggcgttgccttcacctgggtcatggcgctggcctgcgccgcacccccactcgccggctggtccaggtacatccccgagggcctgcagtgctcgtgtggaatcgactactacacgctcaagccggaggtcaacaacgagtcttttgtcatctacatgttcgtggtccacttcaccatccccatgattatcatctttttctgctatgggcagctcgtcttcaccgtcaaggaggccgctgcccagcagcaggagtcagccaccacacagaaggcagagaaggaggtcacccgcatggtcatcatcatggtcatcgctttcctgatctgctgggtgccctacgccagcgtggcattctacatcttcacccaccagggctccaacttcggtcccatcttcatgaccatcccagcgttctttgccaagagcgccgccatctacaaccctgtcatctatatcatgatgaacaagcagttccggaactgcatgctcaccaccatctgctgcggcaagaacccactgggtgacgatgaggcctctgctaccgtgtccaagacggagacgagccaggtggccccggcctaaccaagaaagcttaagtttaaaccgctgatcagcctcgactgtgccttctagttgccagccatctgttgtttgcccctcccccgtgccttccttgaccctggaaggtgccactcccactgtcctttcctaataaaatgaggaaattgcatcgcattgtctgagtaggtgtcattctattctggggggtggggtggggcaggacagcaagggggaggattgggaagacaatagcaggcatgctggggatgcggtgggctctatggc

SEQ ID NO: 26 - DNA, 2716 bp, Artificial Sequence
  Synthetic Construct
acgcgttttctgcagcggggattaatatgattatgaacacccccaatctcccagatgctgattcagccaggaactagttattaatagtaatcaattacggggtcattagttcatagcccatatatggagttccgcgttacataacttacggtaaatggcccgcctggctgaccgcccaacgacccccgcccattgacgtcaataatgacgtatgttcccatagtaacgccaatagggactttccattgacgtcaatgggtggagtatttacggtaaactgcccacttggcagtacatcaagtgtatcatatgccaagtacgccccctattgacgtcaatgacggtaaatggcccgcctggcattatgcccagtacatgaccttatgggactttcctacttggcagtacatctacgtattagtcatcgctattaccacaaatagttatcgagccgctgagccggggggcggggggtgtgagactggaggcgatggacggagctgacggcacacacagctcagatctgtcaagtgagccattgtcagggcttggggactggataagtcagggggtctcctgggaagagatgggataggtgagttcaggaggagacattgtcaactggagccatgtggagaagtgaatttagggcccaaaggttccagtcgcagcctgaggccaccagactgacatggggaggaattcccagaggactctggggcagacaagatgagacaccctttcctttctttacctaagggcctccacccgatgtcaccttggcccctctgcaagccaattaggccccggtggcagcagtgggattagcgttagtatgatatctcgcggatgctgaatcagcctctggcttagggagagaaggtcactttataagggtctggggggggtcagtgcctggagttgcgctgtgggagccgtcagtggctgagctcaactagaagctttattgcggtagtttatcacagttaaattgctaacgcagtcagtgcttctgacacaacagtctcgaacttaagctgcagtgactctcttaaggtagccttgcagaagttggtcgtgaggcactgggcaggtaagtatcaaggttacaagacaggtttaaggagaccaatagaaactgggcttgtcgagacagagaatggatcctggaggcttgctgaaggctgtatgctgaaggagcttacaatctagctggggttttggccactgactgaccccagctagtgtaagctccttcaggacacaaggcctgttactagcactcacatggaacaaatggcccagatctgagactcttgcgtttctgataggcacctattggtcttactgacatccactttgcctttctctccacaggtgtccactcccagttcacaccggcacaatgaatggcacagaaggccctaacttctacgtgcccttctccaatgcgacgggtgtggtacgcagccccttcgagtacccacagtactacctggctgagccatggcagttctccatgctggccgcctacatgtttctgctgatcgtgctgggcttccccatcaacttcctcacgctctacgtcaccgtccagcacaagaagctgcgcacgcctctcaactacatcctgctcaacctagccgtggctgacctcttcatggtcctaggtggcttcaccagcaccctctacacctctctgcatggatacttcgtcttcgggcccacaggatgcaatttggagggcttctttgccaccctgggcggtgaaattgccctgtggtccttggtggtcctggccatcgagcggtacgtggtggtgtgtaagcccatgagcaacttccgcttcggggagaaccatgccatcatgggcgttgccttcacctgggtcatggcgctggcctgcgccgcacccccactcgccggctggtccaggtacatccccgagggcctgcagtgctcgtgtggaatcgactactacacgctcaagccggaggtcaacaacgagtcttttgtcatctacatgttcgtggtccacttcaccatccccatgattatcatctttttctgctatgggcagctcgtcttcaccgtcaaggaggccgctgcccagcagcaggagtcagccaccacacagaaggcagagaaggaggtcacccgcatggtcatcatcatggtcatcgctttcctgatctgctgggtgccctacgccagcgtggcattctacatcttcacccaccagggctccaacttcggtcccatcttcatgaccatcccagcgttctttgccaagagcgccgccatctacaaccctgtcatctatatcatgatgaacaagcagttccggaactgcatgctcaccaccatctgctgcggcaagaacccactgggtgacgatgaggcctctgctaccgtgtccaagacggagacgagccaggtggccccggcctaaccaagaaagcttaagtttaaaccgctgatcagcctcgactgtgccttctagttgccagccatctgttgtttgcccctcccccgtgccttccttgaccctggaaggtgccactcccactgtcctttcctaataaaatgaggaaattgcatcgcattgtctgagtaggtgtcattctattctggggggtggggtggggcaggacagcaagggggaggattgggaagacaatagcaggcatgctggggatgcggtgggctctatggc

SEQ ID NO: 27 - DNA, 2755 bp, Artificial Sequence
  Synthetic Construct
acgcgttttctgcagcggggattaatatgattatgaacacccccaatctcccagatgctgattcagccaggaactagttattaatagtaatcaattacggggtcattagttcatagcccatatatggagttccgcgttacataacttacggtaaatggcccgcctggctgaccgcccaacgacccccgcccattgacgtcaataatgacgtatgttcccatagtaacgccaatagggactttccattgacgtcaatgggtggagtatttacggtaaactgcccacttggcagtacatcaagtgtatcatatgccaagtacgccccctattgacgtcaatgacggtaaatggcccgcctggcattatgcccagtacatgaccttatgggactttcctacttggcagtacatctacgtattagtcatcgctattaccacaaatagttatcgagccgctgagccggggggcggggggtgtgagactggaggcgatggacggagctgacggcacacacagctcagatctgtcaagtgagccattgtcagggcttggggactggataagtcagggggtctcctgggaagagatgggataggtgagttcaggaggagacattgtcaactggagccatgtggagaagtgaatttagggcccaaaggttccagtcgcagcctgaggccaccagactgacatggggaggaattcccagaggactctggggcagacaagatgagacaccctttcctttctttacctaagggcctccacccgatgtcaccttggcccctctgcaagccaattaggccccggtggcagcagtgggattagcgttagtatgatatctcgcggatgctgaatcagcctctggcttagggagagaaggtcactttataagggtctggggggggtcagtgcctggagttgcgctgtgggagccgtcagtggctgagctcaactagaagctttattgcggtagtttatcacagttaaattgctaacgcagtcagtgcttctgacacaacagtctcgaacttaagctgcagtgactctcttaaggtagccttgcagaagttggtcgtgaggcactgggcaggtaagtatcaaggttacaagacaggtttaaggagaccaatagaaactgggcttgtcgagacagagaaaaacctaacccccatggttggcgagggactgctgtgtgtgaaatggtaactgccctcaaggagcttacaatctagctgggggtaaatgacttgcacatgaacacaactagactgtgagcttctagagggcagggaccttaccctagtcatctctcttctcaccctgcacaccctccctgagggatctcatgactcttgcgtttctgataggcacctattggtcttactgacatccactttgcctttctctccacaggtgtccactcccagttcacaccggcacaatgaatggcacagaaggccctaacttctacgtgcccttctccaatgcgacgggtgtggtacgcagccccttcgagtacccacagtactacctggctgagccatggcagttctccatgctggccgcctacatgtttctgctgatcgtgctgggcttccccatcaacttcctcacgctctacgtcaccgtccagcacaagaagctgcgcacgcctctcaactacatcctgctcaacctagccgtggctgacctcttcatggtcctaggtggcttcaccagcaccctctacacctctctgcatggatacttcgtcttcgggcccacaggatgcaatttggagggcttctttgccaccctgggcggtgaaattgccctgtggtccttggtggtcctggccatcgagcggtacgtggtggtgtgtaagcccatgagcaacttccgcttcggggagaaccatgccatcatgggcgttgccttcacctgggtcatggcgctggcctgcgccgcacccccactcgccggctggtccaggtacatccccgagggcctgcagtgctcgtgtggaatcgactactacacgctcaagccggaggtcaacaacgagtcttttgtcatctacatgttcgtggtccacttcaccatccccatgattatcatctttttctgctatgggcagctcgtcttcaccgtcaaggaggccgctgcccagcagcaggagtcagccaccacacagaaggcagagaaggaggtcacccgcatggtcatcatcatggtcatcgctttcctgatctgctgggtgccctacgccagcgtggcattctacatcttcacccaccagggctccaacttcggtcccatcttcatgaccatcccagcgttctttgccaagagcgccgccatctacaaccctgtcatctatatcatgatgaacaagcagttccggaactgcatgctcaccaccatctgctgcggcaagaacccactgggtgacgatgaggcctctgctaccgtgtccaagacggagacgagccaggtggccccggcctaaccaagaaagcttaagtttaaaccgctgatcagcctcgactgtgccttctagttgccagccatctgttgtttgcccctcccccgtgccttccttgaccctggaaggtgccactcccactgtcctttcctaataaaatgaggaaattgcatcgcattgtctgagtaggtgtcattctattctggggggtggggtggggcaggacagcaagggggaggattgggaagacaatagcaggcatgctggggatgcggtgggctctatggc

SEQ ID NO: 28 - DNA, 145 bp, Mus musculus
agaggactaagccacaggtgaggagaaaggggggggggggtctgctgacccagcaacactctttccttctgaggcttaagagctattagcgtaggtgactcagtccctaatcctccattcaatgccctgtgactgcccctgcttc

SEQ ID NO: 29 - DNA, 364 bp, Cytomegalovirus
actagttattaatagtaatcaattacggggtcattagttcatagcccatatatggagttccgcgttacataacttacggtaaatggcccgcctggctgaccgcccaacgacccccgcccattgacgtcaataatgacgtatgttcccatagtaacgccaatagggactttccattgacgtcaatgggtggagtatttacggtaaactgcccacttggcagtacatcaagtgtatcatatgccaagtacgccccctattgacgtcaatgacggtaaatggcccgcctggcattatgcccagtacatgaccttatgggactttcctacttggcagtacatctacgtattagtcatcgctattacca

SEQ ID NO: 30 - DNA, 66 bp, Artificial Sequence
  Synthetic Construct
tttctgcagcggggattaatatgattatgaacacccccaatctcccagatgctgattcagccagga